European Patent Specification EP 3 681 910 B1, published January 25, 2023. Title: INTERLEUKIN-10 RECEPTOR-2 PEPTIDES, ANTIBODIES, COMPOSITIONS, AND METHODS OF USE THEREOF. Applicant: Wisconsin Alumni Research Foundation Cook, Mark Arendt, Maria K. The sequence listing filed with the application follows.

SEQUENCE LISTING (38 sequences)

SEQ ID NO: 1 - protein, 8 aa, artificial
  IL-10 R2 peptide
  variant (1)..(1): X1 is I or V
  variant (3)..(3): X3 is P or K or V or E
  variant (5)..(5): X5 is E or K or R or Q
  variant (7)..(7): X7 is A or V
XPXPXNXR

SEQ ID NO: 2 - protein, 8 aa, artificial
  IL-10 R2 peptide
  variant (1)..(1): X1 is S or L or V
  variant (5)..(5): X5 is A or P
  variant (6)..(6): X6 is K or Q
  variant (7)..(7): X7 is G or T or E
  variant (8)..(8): X8 is N or T or D
XPAFXXXX

SEQ ID NO: 3 - protein, 7 aa, artificial
  IL-10 R2 peptide
  variant (3)..(3): X3 is G or T or Q or V
  variant (4)..(4): X4 is V or T or A
  variant (5)..(5): X5 is R or H ot T or S
  variant (6)..(6): X6 is G or N or K
  variant (7)..(7): X7 is GN or NHP or SAA
PPXXXXX

SEQ ID NO: 4 - protein, 8 aa, Homo sapiens
VPPPENVR

SEQ ID NO: 5 - protein, 8 aa, Canis lupus
VPPPKNVR

SEQ ID NO: 6 - protein, 8 aa, Felis catus
VPPPENVR

SEQ ID NO: 7 - protein, 8 aa, Bos taurus
VPPPENVR

SEQ ID NO: 8 - protein, 8 aa, Ovis aries
IPPPENVR

SEQ ID NO: 9 - protein, 8 aa, Capra hircus
IPPPENVR

SEQ ID NO: 10 - protein, 8 aa, Equus caballus
VPPPENVR

SEQ ID NO: 11 - protein, 8 aa, Sus scrofa
VPPPENVR

SEQ ID NO: 12 - protein, 8 aa, Rattus norvegicus
IPPPEKVR

SEQ ID NO: 13 - protein, 8 aa, Rattus norvegicus
IPPPENVR

SEQ ID NO: 14 - protein, 8 aa, Gallus Gallus
VPKPRNAR

SEQ ID NO: 15 - protein, 8 aa, Meleagris gallopavo
VPKPRNAR

SEQ ID NO: 16 - protein, 8 aa, Danio rerio
VPVPENVR

SEQ ID NO: 17 - protein, 8 aa, Xenopus tropicalis
VPEPQNVR

SEQ ID NO: 18 - protein, 8 aa, Homo sapiens
SPAFAKGN

SEQ ID NO: 19 - protein, 8 aa, Canis lupus
LPAFPKGT

SEQ ID NO: 20 - protein, 8 aa, Felis catus
VPAFPKGN

SEQ ID NO: 21 - protein, 8 aa, Bos taurus
SPAFPKGN

SEQ ID NO: 22 - protein, 8 aa, Ovis aries
SPAFPKGN

SEQ ID NO: 23 - protein, 8 aa, Capra hircus
SPAFPKGN

SEQ ID NO: 24 - protein, 8 aa, Equus caballus
SPAFPKGD

SEQ ID NO: 25 - protein, 8 aa, Sus scrofa
SPAFPQGD

SEQ ID NO: 26 - protein, 8 aa, Mus musculus
VPAFPKTN

SEQ ID NO: 27 - protein, 8 aa, Rattus norvegicus
VPAFPKEN

SEQ ID NO: 28 - protein, 8 aa, Gallus Gallus
PPGVRKGN

SEQ ID NO: 29 - protein, 8 aa, Meleagris gallopavo
PPTVHKGN

SEQ ID NO: 30 - protein, 9 aa, Danio rerio
PPQTTNNHP

SEQ ID NO: 31 - protein, 9 aa, Xenopus tropicalis
PPVASGSAA

SEQ ID NO: 32 - protein, 8 aa, gallus gallus
PGRDAPSD

SEQ ID NO: 33 - protein, 8 aa, gallus gallus
GTNSPWTA

SEQ ID NO: 34 - protein, 8 aa, gallus gallus
TNAFSPQE

SEQ ID NO: 35 - protein, 8 aa, gallus gallus
RTVKYDDI

SEQ ID NO: 36 - protein, 8 aa, gallus gallus
ISSSGSTD

SEQ ID NO: 37 - protein, 8 aa, gallus gallus
HHRHSPAT

SEQ ID NO: 38 - protein, 8 aa, gallus gallus
ADTVIGPP